European Patent Application EP 4 309 659 A1, published January 24, 2024. Title: COMPLEX FOR TREATING OPTIC NERVE DISEASE, AND PREPARATION METHOD THEREFOR AND USE THEREOF. Applicant: CHENGDU GENREZE GENE TECHNOLOGY CO., LTD. The sequence listing filed with the application follows.

SEQUENCE LISTING (6 sequences)

SEQ ID NO: 1 - DNA, 63 bp, artificial sequence
  S1
atttatcacccgccatagtagacgtatcaccaggcagttgagacgaacattcctaagtctgaa

SEQ ID NO: 2 - DNA, 63 bp, Artificial Sequence
  S2
acatgcgagggtccaataccgacgattacagcttgctacacgattcagacttaggaatgttcg

SEQ ID NO: 3 - DNA, 63 bp, Artificial Sequence
  S3
actactatggcgggtgataaaacgtgtagcaagctgtaatcgacgggaagagcatgcccatcc

SEQ ID NO: 4 - DNA, 63 bp, Artificial Sequence
  S4
acggtattggaccctcgcatgactcaactgcctggtgatacgaggatgggcatgctcttcccg

SEQ ID NO: 5 - RNA, 22 nt, Artificial Sequence
  miR-22
aagcugccaguugaagaacugu

SEQ ID NO: 6 - DNA, 90 bp, Artificial Sequence
  S3-miR22-3p
aagcugccaguugaagaacugutttttactactatggcgggtgataaaacgtgtagcaagctgtaatcgacgggaagagcatgcccatcc